European Patent Application EP 4 582 542 A1, published July 9, 2025. Title: Method for Preparing Oligonucleotide with RNA Ligase. Applicant: Asymchem Laboratories (Tianjin) Co., Ltd. The sequence listing filed with the application follows.

SEQUENCE LISTING (60 sequences)

SEQ ID NO: 1 - protein, 203 aa, Diplonema papillatum
MPLSQGAALIRSPTVTAEEKVDGSNLAVYLDASGAVTCQNRGKFVTPSSGSQWGGQLATWLESHYCELVSLLRQRYILYGEWLLARHSIRYQSLPDYFVAFDVYDRTARRFLSAKKRNAFLSQSTIPVVKPLAVGPFAEADILRLLGSPSRYGAAKVEGIYLRSDSGAWLQQRAKVVNSDFLQTIDDDGHWQKRVLEKNQLKY

SEQ ID NO: 2 - protein, 553 aa, Autographa californica nucleopolyhedrovirus
MVYICIDTGSHAKGYAVESSDTDYHIYTKCDRETFEKFIDNKELLKNRHAKDESGNDVKYVDLYTGLIGILTGKSPELSMFSKREDFKDKYGIENLQLYEFVTKLMTVSMVKIIYTLMRYKILNNAKGLLQLMFNYVYVEYYLDYKRAPKSTKILNMLFNVGDEIKITMDKNNQLVVNDLNVLDLNKNNGGYKIDETLTLFVKNVKLLKLYVKLMQRGEYQQEWTEYFQQWKQQLQDRLHHVPEPPERTDIRHNIVMYALNERGPVMPEDENKIVYQIYPSVSHLDQGKKGTLADKEIIVQEKLDGCNFRIICNQNKITYGSRNTYRPDGNFMNYYRIRKDLETCMRSLQARFNDGFIVYGELMGWKDDAKTTPINVINYVDQKESLKYYAYEIQLYGGEFVPFVEAQELLTNVGFNTIPCHKYLYNDFVERLNFKSLMFPQSPLEGFIIRCGNLIYKLKSDYKDLNKLKIEKGPFEWLTCDYIKSNCDAIDKSDMMKILIFCYNMCKVKNYNEKLLFNKVFNLFRQQFNLNHNDYKNLYKQYVNMCKCTEYK

SEQ ID NO: 3 - protein, 334 aa, Shigella flexneri
MFKKYSSLENHYNSKFIEKLYSLGLTGGEWVAREKIHGTNFSLIIERDKVTCAKRTGPILPAEDFFGYEIILKNYEDSIKAVQDIMETSAVVSYQVFGEFAGPGIQKNVDYGDKDFYVFDIIVTTESGDVTYVDDYMMESFCNTFKFKMAPLLGRGKFEELIKLPNDLDSVVQDYNFTVDHAGLVDANKCVWNAEVKGEVFTAEGYVLKPCYPSWMPNGNRVAIKCKNSKFSEKKKSDKPIKAKVELSEADNKLVGILACYVTLNRVNNVISKIGEIGPKDFGKVMGLTVQDILEETSREGITLTQADNPSLIKKELVKMVQDVLRPAWIELVS

SEQ ID NO: 4 - protein, 381 aa, Methanothermobacter thermautotrophicus str. Delta H
MNSMNSDIPFDLIQERTGVPSSRLKVAFARGSLRLLESAGMQALLFKKPLGDLEAGTVIYLGDETEVIRGFPKIRRTLLLSPTIQEHFRDRVAVEEKMNGYNVRIACLSSGETVALTRGGHVCPFTTRKAQELLDLSEFFREHPDLVICGEMIGRDNPYVSQDYPEVGPLGFRVFDLREKNTNRPLPVEERRALLDSYGLPNVRLFGVYPIEEAASEVADIIRALGMAGREGVVMKDPSMEVPPLKYTSSQAHARELAYAFSYPFDFGRPFFFSRVIREGFQAYELDESDDETRERARRLGEAIIYPMLERIKSISAGEAAYEDTVIDVEDREAAEEFIRHLVRLGVSATLADYRDGRATIRRFYQSTTDRINNYLKGGLY

SEQ ID NO: 5 - protein, 379 aa, Pyrococcus abyssi
MVSSVYKEILVKLGLTEDRIETLEMKGGIIEDEFDGIRYVRFKDSAGKLRRGTVVIDEEYVIPGFPHIKRIINLRSGIRRIFKRGEFYVEEKVDGYNVRVVMYKGKMLGITRGGFICPFTTERIPDFVPQEFFKDNPNLILVGEMAGPESPYLVEGPPYVKEDIQFFLFDVQEIKTGRSLPVEERLKIAEEYGINHVEVFGKYTKDDVDELYQLIERLSKEGREGIIMKSPDMKKIVKYVTPYANINDIKIGARVFYELPPGYFTSRISRLAFYLAEKRIKGEEFERVAKELGSALLQPFVESIFDVEQEEDIHELFKVRVKRIETAYKMVTHFEKLGLKIEIVDIEEIKDGWRITFKRLYPDATNEIRELIGGKAFVD

SEQ ID NO: 6 - protein, 440 aa, Naegleria gruberi
MSDSEVNQEAKPEVKPEVKPETHINLKVSDGSSEIFFKIKKTTPLRRLMEAFAKRQGKEMDSLRFLYDGIRIQADQTPEDLDMEDNDIIEAHREQIGGATYMGVRKLATIRTAGEITPIAGAEAIECCHVDGWTCVIKKGEFKQGDRGVYFEIDSFIKEDNDRYPMLSKQVIDYEGQRGTRLRTARLRGQLSQGLFLPMDRFPELASNQVGDDVTEILGITKWEPPISTNLSGEILGEFPTFISKTDQERVQNLIPQIEENKGQKFEVTVKLDGSSMTVYRKDDHIGVCGRNWELRETATNAQWHAARRNKMIEGLQFLNRNLALQGEIIGESIQGNLEKLKGQDFYLFDIYDIDKAQYLTPIERQSLVKQLNDNGFTVKHVPILDDLELNHTAEQILAMADGPSLNKNVKREGLVFKRLDGKFSFKAISNAYLEKHKDR

SEQ ID NO: 7 - protein, 342 aa, Deinococcus radiodurans
MAERQVIKERAQLFPHPNAERLELCKVGTFQLVVRKGEYRDGDPIVIAPEKAVLPPQLAGLYTNADTGASYLHGAEKNRVGSVRLRGEVSQGVILPLDGLEDAPFGEDLAERLGITFWEPPVPVSMAGEVEPRPPAQHYKHHDVEQFGIYVSEFASGEEVMVTEKLHGTQGVYFRTAEGRWLVTSKGLSRGGLTLREAASNVYWQAARNSNLFAEADAAFSGGEVQIFGEVVPVQKGFSYGQHKPTVFVFKVVYDGLRLPRRDWPQWVLDHAVPVLYEGPFDEATVRKLRGGLETVSGKGLHIREGVVVAPKVPRFAADGSDLSVKLISDAYAKKETGEEYS

SEQ ID NO: 8 - protein, 434 aa, Dictyostelium discoideum AX4
MMENIEETLKLVEITDTTTTTTNTTTTNNQEVIIINEKKEIIINENDIEEGRDLDNESGRSLAYFERILKLEAIVGADVIEIATVLGWRVVVKKGLYKVGDPVVYCEIDSILPPWQYFIDDKMDSRGFKIKTIKLRGEISQGYCIPIKELINHPHKKIKAVYKEEEDNNNETIVHLLDEDSNEKIPIEMGRNLTDFIGIKKITEYVQIPRNVNGSNRKAYTFPSFIKRTDQTRIQSVPHYFDLHQDLLWEVTEKLEGSSITVFKKGKESGVCSRNFLIEDFQGSDIHQAVIEDLDLLNRLSTIDLNIALQGEILGPKIQGNIYQLRKNYFKIFDIFLIDSQRYATHDERIEILNSLKLTPSDHMAPVISNSFSLKGKTLSDILDMANGFSILKESKPKILREGLVFKSTSTIGSVNQSVVSFKAISNQYLLKKK

SEQ ID NO: 9 - protein, 338 aa, Gibberella zeae
MPRKLVTVRHISAITPIPGADRIESATVDGWTCVVSTNAFKPGDSGVYFEIDSLLPASDPRFAFLAPKIVSPNGPSHTPDVRVRTVKIRGVLSQGLLMPLNDFPEIVSRLDTIGSDELQDIGFEDTLNVRKYDGPATPLSQDSSLGTPLPDFPSFIPRTEQERVQNLPDVFSTHGSEIFQESTKMDGSSMTIENHPRSQPLFYATARALGLHQTLAKIGRNVAIQGELCGSSVQSNLEGFAIGTHSFFLFAVYDIDDQRYLPPKEVHEIWAPLLGVKHVPVHGYRALNQVGSAVTDLVARAEGKGVNGRKREGIVFKRDDGLFSFKAISNSYLLKHGE

SEQ ID NO: 10 - protein, 362 aa, Neurospora crassa
WTVVGFTSQMNRFKIGDLVVFMEIDSFIPRIDRYWELWSSMDDVFNGEIGLRVRSREVSGTYSQGMIFSLADFPEIVLHHQNRIQKIGKDEATRELLSYSFADSLGIKKWEYPTHVRPVTGIIGELSPLIQRPGNYRIQDIGNNVFNTHAAKNRIYQVTEKLDGVTMHVYKVSNQSPDLLAYFPALKPTAGSIPIPPTMQTPRGRVGVCNRKHEFFDDGKNIYWETAKTSGILDKIHKIPYRNIAIQGELVGSHIQGNTMQYPEGKHEFVVFGIWDMDARDYLATKSVELLCKTLDIAHVPVLGYGPVTKYGKSVEEILAYADKLGPGEYGGVKEGLIFRANDDWKKGFKVISNGWLKMTGK

SEQ ID NO: 11 - protein, 428 aa, Pyricularia oryzae 70-15
MEGDSPVVAVTSPTIPTDSTLAVSPTAEKAASTESFSAPAVRKLVTLRRISRIRPVKNAKLPKSKYVAITVDGWEVVVNAKRDQRRFREGQLVVFFQIDSFVPENDGNFWEEMSTSAELFQERRGFRIGTLRIGESSLISQGRVFHLGEYPRVEEVVAELQKVHGDKDGLEVAMQRSFDDVLGVVKWDVPEEHKGAHYGPPPPMIPRTALNRIQDVTQQLWERHAATRVQITEKLDSCPISIYFVRNDSPFAKCLPALHDFAGKPDAQRRQQQLCVFPHGRVGVCANRLEYVCAPGQRFWAVVERLGIPGRLAREGRTAVVQGELVAPDRGGPGGFYAFSLWTEGGKHGGFDGEETQRAALRRMGVPLVPLVGYRAIGEFASSTGEMLAKADGRGFRGQLREGFVLKNVKENIWVKVISNAWLEWYEE

SEQ ID NO: 12 - protein, 334 aa, Shigella phage pSs-1
MFKKYSSLENHYNSKFIEKLYSLGLTGGEWVAREKIHGTNFSLIIERDKVTCAKRTGPILPAEDFFGYEIILKNYADSIKAVQDIMETSAVVSYQVFGEFAGPGIQKNVDYGDKDFYVFDIIVTTESGDVTYVDDYMMESFCNTFKFKMAPLLGRGKFEELIKLPNDLDSVVQDYNFTVDHAGLVDANKCVWNAEAKCEVFTAEGYVLKPCYPSWLPNRNRVAIKCKNSKFSEKKKSDKPIKAKVELSEADNKLVGILACYVTLNRVNNVISKIGEIGPKDFGKVMGLTVQDILEETSREGITLTQADSPSLVKKELVKMVQDVLRPAWIELVS

SEQ ID NO: 13 - protein, 347 aa, Buttiauxella phage vB_ButM_GuL6
MFVKYSSLTNHYEGKFINGVIMNGLTGGVWVAREKIHGANFSLITSDGEKVIPAKRSGEILPTEQFYGCEPVVARYAPAIRKLWDVINTAQQVSGIYVDSLVIQVYGEFAGRGVQKDVDYGEKDFYVFDIRVNGEFLHDNIVAVYAKSVGLKMAPLLAYGTFDEIRALPITFDSVVNLANSGAIPAHNGVEPEFKNFMTLKDGEGENIAEGFVMKPVHPAFMPNGERVAIKCKTTKFSEKKNKQANRFNAPAELSENDKAKLDVFTCYLTENRVKNVLSKIDSANLTAKDFGRVMGLTVQDALEEIERNYGPFIEQFENPTLAKKTFTNEASSLIRTNWGAILNNEF

SEQ ID NO: 14 - protein, 416 aa, Trypanosoma brucei gambiense DAL972
MLRCLGVRHFRRTPLLFVGGDGSIFERYTEIDNSNERRINALKGCGMFEDEWIATEKVHGANFGIYSIEGEKMIRYAKRSGIMPPNEHFFGYHILIPELQRYVTSIREMLCEKQKKKLHVVLINGELFGGKYDHPSVPKTRKTVMVAGKPRTISAVQTDSFPQYSPDLHFYAFDIKYKETEGGDYTTLVYDEAIELFQRVPGLLYARAVIRGPMSKVAAFDVERFVTTIPPLVGMGNYPLTGNWAEGLVVKHSRLGMAGFDPKGPTVLKFKCTAFQEISTDRAQGPRVDEMRNVRRDSINRAGVQLPDLESIVQDPIQLEASKLLLNHVCENRLKNVLSKIGTEPFEKEEMTPDQLATLLAKDAMKDFLKDTEPSIVNIPVLIRKDLTRYVIFESRRLVCSQWKDILKRQSPDFSE

SEQ ID NO: 15 - protein, 332 aa, Klebsiella phage vB_Kpn_F48
MFEKYSSLENHYNNRFIEKIRHHGYDVTEGWCAREKIHGTNFSIIIERDAVTCAKRTGPILPAEDFFGYTVILKKYNDSIKAVQHTIKEGSSMQIFGEFAGSGIQKGVDYGEKDFYVFDILVKTDKGTHQFVDDFMMEQMCCTFGFKVAPLMGRGSFDELAKLPNEFQINVNRYNEAAEVDLRNANTRVWPAEEATDNTAEGYVLKPNYPRFLANGSRVAIKCKNSKFSEKAKSDKPIKPKAVLSEIDQEVLQKFSEYVTIQRVNNVISKIGQVGPKDFGKVMGLTVQDILVEAGREGLEVIQAEQPDIVKKEITKLVQDVLRPAWIELVSN

SEQ ID NO: 16 - protein, 487 aa, Pyrococcus horikoshii OT3
MVVPLKRIDKIRWEIPKFDKRMRVPGRVYADEVLLEKMKNDRTLEQATNVAMLPGIYKYSIVMPDGHQGYGFPIGGVAAFDVKEGVISPGGIGYDINCGVRLIRTNLTEKEVRPRIKQLVDTLFKNVPSGVGSQGRIKLHWTQIDDVLVDGAKWAVDNGYGWERDLERLEEGGRMEGADPEAVSQRAKQRGAPQLGSLGSGNHFLEVQVVDKIFDPEVAKAYGLFEGQVVVMVHTGSRGLGHQVASDYLRIMERAIRKYRIPWPDRELVSVPFQSEEGQRYFSAMKAAANFAWANRQMITHWVRESFQEVFKQDPEGDLGMDIVYDVAHNIGKVEEHEVDGKRVKVIVHRKGATRAFPPGHEAVPRLYRDVGQPVLIPGSMGTASYILAGTEGAMKETFGSTCHGAGRVLSRKAATRQYRGDRIRQELLNRGIYVRAASMRVVAEEAPGAYKNVDNVVKVVSEAGIAKLVARMRPIGVAKGAAALEH

SEQ ID NO: 17 - protein, 372 aa, Enterobacteria phage RB69
MEKLYYNLLSLCKSSSDRKFFYSDDVSPIGKKYRIFSYNFASYSDWLLPDALECRGIMFEMDGETPLRIASRPMEKFFNLNENPFTLSIDLNDVKYLMTKEDGSLVSTYLDGNMVRFKGSIKSDQAASATSILLDINHKDLADRLLELCNDGFTANFEYVAPSNKIVLTYPEKRLILLNIRDNNTGKYIEYDDIYLDPVFRKYLVDRFEAPEGDWVPGVKSSTNIEGYVAVMKDGSHFKLKTDWYVALHTTRDSISSPEKLFLAIMNGASDDLKAMYADDEFSFKKVELFEKAYLDFLDRSFYICLDAYDKHKGKDRKTYAIEAQAICKGAQSPWLFGIIMNLYQGGSKEQMMTALESVFIKNHKNFIPEGY

SEQ ID NO: 18 - protein, 269 aa, Aeromonas virus Aeh1
MIVGRYEKQIRQLHKCLVHLDMIDKEDSIGVFGEYAGIMSYGKWIQTGIEYGPQDFYVFDIIVQPLDGDQFMLEDLQVEELCKALGLKTAPLLKVGTFADIMKIPVDLQSVVMEVNAGKPIDIRVGTDNIAEGYVAKPNVPARFKNGNRVAIKCKNEKWSETGKGRAVQVEVKELSEKDKALVLDITRYITDNRLKNVLSKMDTPKTSEFGKVLGLMSKDVQKDYERDELDGVSVKEATDEAGRVMRMINTEIGNMIRPNWVSICDGDW

SEQ ID NO: 19 - protein, 374 aa, Escherichia phage UFV-AREG1
MQELFNNLMELCKDSQRKFFYSDDVSASGRTYRIFSYNYASYSDWLLPDALECRGIMFEMDGEKPVRIASRPMEKFFNLNENPFTMNIDLNDVDYILTKEDGSLVSTYLDGDEILFKSKGSIKSEQALMANGILMNINHHQLRDRLKELAEDGFTANFEFVAPTNRIVLAYQEMKIILLNIRENETGEYISYDDIYKDAALRPYLVERYEIDSPKWVEEAKNAENIEGYVAVMKDGSHFKIKSDWYVSLHSTKSSLDNPEKLFKTIIDGASDDLKAMYADDEYSYRKIEAFETTYLKYLDRALFLVLDCHNKHCGKDRKTYAMEAQGVAKGAGMDHLFGIIMSLYQGYDSQEKVMCEIEQNFLKNYKKFIPEGY

SEQ ID NO: 20 - protein, 339 aa, Klebsiella phage KP27
MFKKYSSLTNHYEGKFINGVIMNGLTGGVWVAREKIHGANFSFITDDGITVTPAKRTDVVKPAEDFYGCSAVVAKYSPGIRKMWETLKKTGTYDDLVIQVYGEFAGRGVQKDVDYGEKDFYVFDIRVNGEFLPDNLCSLISRSHGLKMAPLLGYGTFEEIKELPITFESVVNKANSGIGSDNTVYGEFVYPIMDVEEGNIAEGFVMKPVSPAFMPNGERVAIKCKTTKFTEKKAKKATRFNAPVSLSEKDKNQLDEFVCYLTENRVKNVLSKLDLASITAKDFGRIMGLTVQDAIEEISRNHGPFLEQFEDPAMAKKLFVTEAQNMIRPVWGKILNHEF

SEQ ID NO: 21 - protein, 370 aa, Fusarium proliferatum
MPRKLVTVRHVSAITAIPRADRIAAATVDGWTCVVPTNIFKAGDRAVFFEIDSLLPATDPRFAPLAPKIIGPGGPTSAPDIRVQTIQIRGVLSQGLLLPLADFPEIVAKLDGIPSDKLRDISFEDILNVRKFEKPAIPLHQTSTSDAPLPEYPDFIPRTNQERVQNLTDVFSEHGTEIFEESTKMDGSSTTVFYLNDGNPLAKTVPSETRHNGVAVCSRNRILVENHPRSPPLFYATARALNLHEKLPKIGRNIALQGELCGSSIQSNFEGFLKGTHCFFLFAVYDIDEQRYLPPREVYERWAPLLGVEHVPVHGYRPLNEMGSQITDLVDRAEGRGINGRKREGIVFKREDGQFSFKAISNSYLLTHGE

SEQ ID NO: 22 - protein, 380 aa, Thermococcus barophilus
MVSLHFKHILLKLGLDKERIEILEMKGGIVEDEFEGLRYLRFKDSAKGLRRGTVVFNESDIILGFPHIKRVVHLRNGVKRIFKSKPFYVEEKVDGYNVRVAKVGEKILALTRGGFVCPFTTERIGDFINEQFFKDHPNLILCGEMAGPESPYLVEGPPYVEEDIQFFLFDIQEKRTGRSIPVEERIKLAEEYGIQSVEIFGLYSYEKIDELYELIERLSKEGREGVVMKSPDMKKIVKYVTPYANVNDIKIGSRIFFDLPHGYFMQRIKRLAFYIAEKRIRREDFDEYAKALGKALLQPFVESIWDVAAGEMIAEIFTVRVKKIETAYKMVSHFERMGLNIHIDDIEELGNGYWKITFKRVYDDATKEIRELWNGHAFVD

SEQ ID NO: 23 - protein, 420 aa, Trypanosoma brucei
MDQSDFSPYIEIDLPSESRIQSLHKSGLAAQEWVACEKVHGTNFGIYLINQGDHEVVRFAKRSGIMDPNENFFGYHILIDEFTAQIRILNDLLKQKYGLSRVGRLVLNGELFGAKYKHPLVPKSEKWCTLPNGKKFPIAGVQIQREPFPQYSPELHFFAFDIKYSVSGAEEDFVLLGYDEFVEFSSKVPNLLYARALVRGTLDECLAFDVENFMTPLPALLGLGNYPLEGNLAEGVVIRHVRRGDPAVEKHNVSTIIKLRCSSFMELKHPGKQKELKETFIDTVRSGALRRVRGNVTVISDSMLPQVEAAANDLLLNNVSDGRLSNVLSKIGREPLLSGEVSQVDVVLMLAKDALKDFLKEVDSLVLNTTLAFRKLLITNVYFESKRLVEQKWKELMQEEAAAQSEAIPPLSPAAPTKGE

SEQ ID NO: 24 - protein, 400 aa, Trypanosoma brucei gambiense DAL972
MVGGDGSIFERYTEIDNSNERRINALKGCGMFEDEWIATEKVHGANFGIYSIEGEKMIRYAKRSGIMPPNEHFFGYHILIPELQRYVTSIREMLCEKQKKKLHVVLINGELFGGKYDHPSVPKTRKTVMVAGKPRTISAVQTDSFPQYSPDLHFYAFDIKYKETEGGDYTTLVYDEAIELFQRVPGLLYARAVIRGPMSKVAAFDVERFVTTIPPLVGMGNYPLTGNWAEGLVVKHSRLGMAGFDPKGPTVLKFKCTAFQEISTDRAQGPRVDEMRNVRRDSINRAGVQLPDLESIVQDPIQLEASKLLLNHVCENRLKNVLSKIGTEPFEKEEMTPDQLATLLAKDALKDFLKDTEPSIVNIPVLIRKDLTRYVIFESRRLVCSQWKDILKRQSPDFSE

SEQ ID NO: 25 - protein, 334 aa, Escherichia phage JS98
MFKKYSSLENHYNSKFIEKLRTNGLTGGEWVAREKIHGTNFSLIIERDAVTCAKRTGPILPAEDFYGYEIVLKNYADSIKSVQHLIESINYQSYQIYGELAGPGIQKNVDYGDKDFYVFDIRVTKEDGTESVLTDTLMEAFCIIHKFKVAPCLATGSFEDLIKLPNDFDSVIPDYNFAVDNAGLTIANSTDFIPKVEGKVFTAEGFVLKPDIPTWLPNGNRVAIKCKNSKFSEKKKSDKPIKAAVVLSQDDMDLMWQFTDYVTVNRINNVISKIGEVSKKDFGKVMGLTVQDILEEAAREELELTDAENPVEVKKQLVECVKDTLRAVWIELVS

SEQ ID NO: 26 - protein, 365 aa, Variovorax gossypii
MVPGLFSFCVTINHREKTTMRKLVTVRTVDFVRPIPGADAIECAVVEGWSVVIKKGEFAVGDRCVFFEIDAFLPLDDPRFAFLEKAAITWNEQRGVRLRTMKLRGQISQGLILPLSQFPEIDALALADPDLRHRDWAELLGIGKWEPVIPACLSGEVEGPFPSFISKTDQERIQNLPEVLAANDGLAFEVTVKLDGSSMTVFHNAGAVGVCGRNWQLRETPGNSLWRVAREDRLLEVLATLGRNLALQGEIIGEGIQGNPEKLRGQQFHVFDVFDIDRGAYCGMDERNAVIDALRVLGATVRSVPLLEVAALDRFDGSMAGVLAYAEGPSLNPGTSREGVVFKRLDGGLSFKAISNTYLLKHADR

SEQ ID NO: 27 - protein, 342 aa, Undibacterium pigrum
MRKLVTIRTVSNIRPIPDADAIECASVDGWSVVVKKNEFQVGDACVYFEIDSFLPLSDARFAFLEKNKIIWNEKNGIRLRTIKLRGQISQGMILPLNQFPELIELTDDGNADFSQVLGIEKWEPAIPASLSGEVEGAFPEYIRKTDQERIQNLTEVLSTQAQEEFEVTIKLDGSSMTVFHNAGVSGVCGRNWWIRESEANSLWRVAKQNQMLTALTAFGRNLALQGEIIGEGIQGNPEKMRGQDFYLFDIFDIDASRYLGRAERQEVLAALRALGATVHEVPWLENMTLERFAGDVSKVLDYAEGGSLNPATAREGVVFKRLDGSMSFKAISNTYLLKHGDR

SEQ ID NO: 28 - protein, 338 aa, Panteoa phage Phynn
MFVKYSSLTNHYEGKFINGIVMNGLASGEWVAREKIHGANFSFLTCDGATVIPAKRSGEILPGERFYDCENVVAKYLESVRNLWQKLFVTGFYDVLNVQIFGELAGRGVQKDVDYGEKDFYVFDIKVNGEYLDDRLVSSLARECGLKMAPLLGYGSYEHLKELPLTFESVVLFSPSRTEVKGEETVHNINEAADDVENIAEGYVLKPVVTAYMTNGSRVAIKCKTSKFSEKKNKSTTAFNAPVSLSEADKLKLGEYVNYLTENRVKNVLSKIDASNLTAKDFGRVAGLTVQDALEEIERNEGDFVTKFENPAFAKKLFVSEAQSLIRPVWGLILNNEF

SEQ ID NO: 29 - protein, 369 aa, Stenotrophomonas phage Marzo
MYLNLQMMRDALGHDETVRFKEETVDGREFVIVSYMIANDDLWSRSFGAEARGITFDKVTGECVSRPFHKFFNVGEKEFTQPVALQNTVWTAYPKIDGSMITPVMVNGKVRLKTKKSFYSNVAREAQANLDPETEGQMAAFLISGWTPIYEYTSPTTKIVVQHDKPAFKLLAGRATQDGHYLTPTDLALHPDAIKPEFHSASINELLYTARDLEGVEGWVLVDHEGGYDRVKIKTDWYNRLHRVLDLRVRDVVEFIRDEKLDDMIPNLLNMGVDMDVIQSIENRVVNAISDAVTHVKTVVLGASGLPLKEAVQFIEKHGGIYVKACHRTWRTGCIEPQMELIVRLYFQYHLQDYELTSIGNPNFGGKDG

SEQ ID NO: 30 - protein, 360 aa, Waterburya agarophytonicola
MELQDYLRNRGLDKLTEEYNIKVNRHSKIDNLVCLKYSQLESPMGEKIVQQCRGIIFDETNNWNIVSYPYDKFFNYGESYAPKLNWDAARIYEKLDGSLMTLFYYEGEWRVQSSGMADAGGDVSGFKYTFQSLFWKVWQELDYQLPTETEYCFMFELMTPYNRIVVRHDRHKLVLHGVRNKVTLKEEDPQIWTDKYNWQLVATYPLQTLEEIVAMTDKLDPMDSEGYIICDREFKRIKVKSPQYVAISHLKTGFSSRRMLEIVVTNEGEEFLNYYPEWQELYQQIATQYNALIEEIEEQYYKYQNIPVQKDFAIAVKNLSYSGILFALRAGKSNSVKESLAQTSIYKLENLLNINFQELG

SEQ ID NO: 31 - protein, 355 aa, Streptomyces avermitilis
MSTLRVTAEVLTIHPHPNADALELAQVGLYRAVVAKGAYRTGETAVYIPEQSVLPAGLIEELGLTGRLAGSGSDRVKAVRLRGELSQGIVCRPKALADVDLARTVADGTDFAELLGITKWVPPIPPTMSGEIESVPDLLRWVDIENIQRYPDIFTPGEPVVLTEKLHGTACLVTYLADEDRVHVSSKGFGAKSLALKEDPRNLYWRAVHGHGVAQAAARLAERLGARRVGIFGEVYGAGVQDLTYGADGRRDTLGYAVFDVSADIDGEVRWLDAADRLDGELPLVPRLYEGPYDIERVLETASGRETVSGHGLHLREGVVIRSATERRSPVTGGRAIAKAVSPAYLTRKGGTEYE

SEQ ID NO: 32 - protein, 374 aa, Escherichia phage p000v
MEKLYYNLLSLCKSSSDRKFFYSDDVSPIGKKYRIFSYNFASYSDWLLPDALECRGIMFEMDGETPLRIASRPMEKFFNLNENPFTLSINLDDVKYLMTKEDGSLVSTYLDGGTVRFKSKGSIKSDQAVSATSILLDIDHKNLADRLLELCNDGFTANFEYVAPTNKIVLSYPEKRLILLNIRDNNTGEYIEYDDIYLDPVFRKYLVDRFEVPEGDWTSDVKSSTNIEGYVAVMKDGSHFKLKTDWYVALHTTRDSISSPEKLFLAIVNGASDDLKAMYADDEFSFKKVELFEKAYLDFLDRSFYICLDTYDKHKGKDRKTYAIEAQAVCKGAQTPWLFGIIMNLYQGGSKEQMMTALESVFIKNHKNFIPEGY

SEQ ID NO: 33 - protein, 349 aa, Fusarium subglutinans
MPRKLVTVRHVSAITAVPRADRIAAATVDGWTWVVPVNVFQVGDRAVFFEIDSLLPATDPRFAPLAPKIIGPGGPTSAPDIKFGGFAELDGIPSYKLRDISFEDILHVRKFEKPAMPLQQTSASETPLPEYPDFIPRTNQERVQNLTDVFSEHGTEIFEESTKMDGSSMTVFYLNDANPLANTVPSEARHNGVSVCSRNRILVENHPRSPSLFYSTARALNLHETLPKIRRNIALQGELCGSSIQSNFEGFPKGTHCFFLFAVYDIDEQRYLPPREVYETWAPLLGVKHVPVHGYRPLNEMGSQITDLVNRAEGRGINGRKREGIVFKREDGQFNFKAISNSYLLTHGE

SEQ ID NO: 34 - protein, 374 aa, Vibrio phage JN02
MEKLYYNLLSLCKSSSDRKFFYSDDVSPIGKKYRIFSYNFASYSDWLLPDALECRGIMFEMDGETPVRIASRPMEKFFNLNENPFTLSINLDDVKYLMTKEDGSLVSTYLDGGTVRFKSKGSIKSDQAVSATSILLDIDHKNLADRLLELCNDGFTANFEYVAPTNKIVLTYPEKRLILLNIRDNNTGEYIEYDDIYLDPVFRKYLVDRFEVPEGDWTSDVKSSTNIEGYVAVMKDGSHFKLKTDWYVALHTTRDSISSPEKLFLAIVNGASDDLKAMYADDEFSFKKVELFEKAYLDFLDRSFYICLDTYDKHKGKDRKTYAIEAQAVCKGAQTPWLFGIIMNLYQGGSKEQMMTALESVFIKNHKNFIPEGY

SEQ ID NO: 35 - protein, 332 aa, Shigella sonnei
MFKKYSSLENHYNSKFIEKLYTNGLTTGVWVAREKIHGTNFSLIIERDNVTCAKRTGPILPAEDFYGYEIVLKKYDKTIKAVQEFMYTARAVSYQVFGEFAGGGIQKGVDYGEKDFYVFDILINTESGDNTYLTDYEMQDFCNEFGFKMAPMLGRGTFDALIMIPNDLDSVLAAYNATASEDLVEANNCVFDANVIGDNTAEGYVLKPCFPKWLPNGTRVAIKCKNSKFSEKKKSDKPVKTQVPLTEIDKNLLDVLACYVTLNRINNVISKIGAVTPKDFGKVMGLTVQDILEETSREGIVLTSSDNPNLVKKELVRMVQDVLRPAWIELVS

SEQ ID NO: 36 - protein, 379 aa, Thelonectria olida
MARKLVTVRRIAALNEIPGADRIEAASVDGWTCVVPVGQFEKGGLAVFFEIDSLLPAKDERFAAFAKTNDGEDIRLKTVRIRKVTSQGLLMPLATFPEIKAVVDKLALELQPAEVEARLRAVSFEKELGVRKFVAPEQASQKGVAGGRPAYMADFPVFIPRTDQERIQNMPGAFDEWPDSVFQETTKMDGSSMTAYFLRRDSPYFDMLPPLPLTAKNAEFPNGRFGVCSRNRDIGEVPNSGLFWPTALANNLPSTLSRLDRNIALQGELCGSSIQANFEGFAPGAHDFFLFTIWDVDKQRPLPPREVHEIWAPKLGVKHVPVVGYHALKYVASSVGELVKRADGKGINGKKREGIVLKHVDGKVSFKAISNSYLLKHGE

SEQ ID NO: 37 - protein, 333 aa, Citrobacter phage Merlin
MFEKYSTLENHYNNKFIERIRSAGFDLTETWVAREKIHGTNFSIIITKDTVTCAKRTGPILEAEDFFGYEIILKKYDKSIKALQDTMKNMTTESYQLFGEFAGGGIQKGVNYGEKDFYVFDCLVKTPGGIVEYSDDYILTAFCNVFGFKMAPLLGRGKFDDLIQMSNMLDVVVNDYNKLAEADLEAANLKVWPVVVSEDNIAEGYVLKPCYPKFFNNGARVAIKCKNSKFSEKSKSDKLIKAKVELTEADKKCLSAFSEYVTINRVNNVISKIGTVTTKDFGRVLGLTMKDILEEAAREEVVLTSADNPDIVKKELTRILQETLRPAWIELIS

SEQ ID NO: 38 - protein, 370 aa, Fusarium albosuccineum
MPRKLVTVRQISAISPITGADRIETATIDGWTCVVPVGDFKPGDRGLYFEIDSLLPGADPRWAFLAPKNGPTPPADIRVKTLRVRGVLSQGLLLPLLSFPEVTAVIDALSPAEIDVKLRDMSFEEVLRVRKYEKPVVPLPNGAPDVTPLPEFPYFVPKTEAERVQNLPDVFISHGDEVFQESTKMDGSSMTVFYLGADSPHHDILDADISSDGVYVCSRNRMLVENHPRSPPLFWSTARALNLPATLSSLGRNIAIQGELCGSSIQSNYEGFGRGEHNFFLFSVWDIDAQRYLPPREVHETWAPRLGVKHVPVHGYRPLKEIGGSVADLVARAEGKGVDGRKREGIVLKQEDGSLSFKAISNSYLLKHGE

SEQ ID NO: 39 - protein, 327 aa, Vibrio phage nt-1
MSFVKYTSLENSYRQAFVDKCDMLGVRDWVALEKIHGANFSFIVEFDGGYTVTPAKRTSIIGATATGDYDFYGCTSVVEAHKEKVELVANFLWLNEYINLYEPIIIYGELAGKGIQKEVNYGDKDFWAFDIFLPQREEFVDWDTCVAAFTNAEIKYTKELARGTLDELLRIDPLFKSLHTPAEHEGDNVAEGFVVKQLHSEKRLQSGSRAILKVKNEKFKEKKKKEGKTPTKLVLTPEQEKLHAEFSCYLTENRLKNVLSKLGTVNQKQFGMISGLFVKDAKDEFERDELNEVAIDRDDWNAIRRSLTNIANEILRKNWLNILDGNF

SEQ ID NO: 40 - protein, 334 aa, Shigella phage SH7
MFKKYSSLENHYNSKFIEKLYSLGLTGGEWVAREKIHGTNFSLIIERDKVTCAKRTGPILPAEDFFGYEIILKNYDDSIKAVQDIMETSAVVSYQVFGEFAGPGIQKNVDYGDKDFYVFDIIVTMESGDVTYVDDYMMESFCNTFKFKIAPLLGRGKFEELIKLPNDLDSVVQDYNFTVDHAGLVDANKCVWNAEAKGEVFTAEGYVLKPCYPSWMPNGNRVAIKCKNSKFSEKKKSDKPIKVKVELSEADNKLVGILACYVTLNRVNNVISKIGEIGPKDFGKVMGLTVQDILEETSREGITLTQADNPSLIKKELVKMVQDVLRPAWIELVS

SEQ ID NO: 41 - protein, 335 aa, Vibrio phage phi-ST2
MSFVKYTSLENSYRQAFVDKCDMLGVKEWVALEKIHGANFSFIVEFKPSTEEVPGEMSVTPAKRTSTIGANAMGDYDFYGCTSVVEAHIEKMQDISNWLFANDFIKNDETIIVYGELAGKGIQKEVNYGDKDFWAYDILCPETGEFLDWDVVLKACKFAGVKTTHEIARGTLDELLKIDPLFRSFHTPADVDSENVAEGFVVKQLKAEKRLHNGSRAILKVKNEKFKEKKNKQGKTPRAKVVLTEEQEKLHAAFSCYLTENRLRNVLSKIGKVEAKQFGMVSGLFVKDAKDEFERDERDEVAIPRDDWDVIKRSLVNVANEILRKNWLNIVDGTF

SEQ ID NO: 42 - protein, 339 aa, Klebsiella phage KP15
MFKKYSSLTNHYEGKFINGVIMNGLTGGVWVAREKIHGANFSFITDDGITVTPAKRTDVVKPAEDFYGCSAVVAKYSPGIRKMWETLKKTGTYDDLVIQVYGEFAGRGVQKDVDYGEKDFYVFDIRVNGEFLPDNLCSLISRSHGLKMAPLLGYGTFEEIKELPITFESVVNKANSGIGSDNTVYGEFVYPIMDVEEGNIAEGFVMKPVSPAFMPNGERVAIKCKTTKFTEKKAKKATRFNAPVSLSEKDKNQLDEFVCYLTENRVKNVLSKLDLASITAKDFGRIMGLTVQDAIEEISRNHGPFIEQFEDPAMAKKLFVTEAQNMIRPVWGKILNHEF

SEQ ID NO: 43 - protein, 335 aa, Escherichia phage JN02
MFKKYSSLENHYNSKFIEKLYTNGLTTGVWVAREKIHGTNFSLIIERDNVTCAKRTGPILPAEDFYGYEIVLKKYDKAIKAVQEVMESISTSVPVSYQVFGEFAGGGIQKGVDYGEKDFYVFDIIINTESDDTYYMSDYEMQDFCNTFGFKMAPMLGRGTFDSLIMIPNDLDSVLAAYNSTASEDLVEANNCVFDANVIGDNTAEGYVLKPCFPKWLSNGTRVAIKCKNSKFSEKKKSDKPVKTQVPLTEIDKNLLDVLACYVTLNRVNNVISKIGTVTPKDFGKVMGLTVQDILEETSREGIVLTSSDNPNLVKKELVRMVQDVLRPAWIELVS

SEQ ID NO: 44 - protein, 346 aa, Yersinia phage JC221
MFKKYSSLTNHYEGKFINGVIMNGLTGGVWVAREKIHGANFSLMTKDGINVIPAKRSGEILPAEQFYGCEPVVAKYSPAIRMIWRWIHDLNVINDAHEDLEIQVYGEFAGRGVQKDVDYGEKDFYVFDIRVNGLFLADNVVANYATGSGLKMAPLLAYGTFEEIKELPITFDSVVNLANSGMVMKSNDFEPEFKNYMTLKDGEGVNIAEGFVMKPVIPAFMPNGDRVAIKCKTTKFTEKKNKQANRFNAPVALSENDKAKLEVFTCYITENRVKNVLSKMDRTNLTAKDFGRVMGLTVQDALEEIERNYGPFLEQFEDPTLAKKTFSNEASNLVRENWGAILNNEF

SEQ ID NO: 45 - protein, 348 aa, Cronobacter phage vB_CsaM_GAP161
MFVKYSSLTNHYEGKFINGVIMNGFTGCVWVAREKIHGANFSLITSDGIKVIPAKRSGEILPAEQFYGCEPVVAKYSEPVRKLWEILANACEYKEYADTGSLVVQVYGEFAGRGVQKDVDYGEKDFYVFDIRVNGEFLPDNVVATYSVAVGLKMAPLLAYGSFDEIRALPITFDSVVNLANSGAIPAKNGVEPEFKNFMTLKDGEGENIAEGFVMKPVQPAFMPNGERVAIKCKTTKFTEKKNKQANRFNAPSELSETDKAKLNEFTCFLTENRVKNVLSKIDSANLTAKDFGRVMGLTVQDALEEIERNYGPFLEQFENPTLAKKTFTNEASNLVRENWGAILNNEF

SEQ ID NO: 46 - protein, 524 aa, Amsacta moorei entomopoxviru
MVYIILDVGSKAKGYDIISSDYDYIIITKSSADIYAEEWIEDNKRLINRHSNKKNNNDITFVDISKAFMGIIKGNYYFLGIYGTKENIKNDMIFYFVRYITKYYISLILKTMTKYQINNTSDREPKNLLALLYNLSYVNYWLKNNDFPVINKLPELLEEDKIELYNILMMKRLNNELATEEQGSIIQDYRKVLLENVNKLEKPKKIKNISNIIMMYLICNKPLYIPEILNNDDEINKIIYPSIKQLNHCKNSLLYGKEIFVQEKLDGCNFRIIYNNGIITFGSRYTYYENKNFMNYYRIKDKLIDCTNKINKFLNLKKFIIYGELIGSYQNDEGINKLIIKNVNYFNDNRIEYYAYEIKNCDNKNKIHFIDFDICQIVLNAAGFNVINYETIKYNDFIENIKYKSIVFNHNDESKVEGYIIRYKNIRYKVKKSYNLTKLTHKNILYNITEESVLNFINNIDINQDNVLYYITKYYKNLIHMNNIDNNVPIYKIFGKIYGFINKKYKFNDNNIYKNKLSEFYKLL

SEQ ID NO: 47 - protein, 364 aa, Chitinophaga sp. S165
MRRLSIYLASIDEINQIRNPKGFTFRSKEMERKLVSPVVIDDIQPIVGADLIEVATVKGWKLVVKKNEFSIGDHAVYCEIDSFLPIREEFEFLRKSSYRKMGEQEGFRLKTMKLRGQISQGLLLPVSLLEGYTYQIGEDVSARLGVIKYEPPVPAALGGIAKGLFPSFMPKTDEERIQNLSGQYEEFRKHTFYVTEKLDGSSATFYLNEGVFGVCSRNLDLEETEDNTFWKIARVEKLEEKLAALGKNFAIQGELIGEGVQGNAYGLRGQTVRFFNAFDIDRYEYLGLDEFKALFASLGLQTVPILDEEYVLPASLDEMLTIADGASVLSPKGKEVEREGLVIRSKDRKISFKVISNKFLLNER

SEQ ID NO: 48 - protein, 351 aa, Candidatus Aminicenantes bacterium
MERKLATIRKVNEIKPIENADMIELAIVDGWQCVVKKGEFKPGDLGVYFEIDSYLPIEERYEFLRKSSYKKIPDQLQGQRAEGFRLKTVKLRGQISQGLMLPLDMFPELKTTSPGSDVTESLNVELYEPPVPANLAGQVRGKLPGFLKKTDEERIQNLPEYFENYKNISFECTEKIDGSSMTVYSTEDDQGVCSRNLNLKEDEQNTLWKIAKQLELHKLLKELNKNLALQGEIAGEGIQKNPLKIKGQHLFLFNIWDIEKRQHLTPEERMEIFDSFEKRVPIRHVPVISSEIKVFEKYKTMQELLDFAVGKSLLNKDIGREGIVLKSLESIGREIISFKVISNKYLLKHNA

SEQ ID NO: 49 - protein, 327 aa, Massilia rubra
MRKLATVRKVIDIAPIPGADAIECVTVDGWKVVSKKGEFQIGGNALYLEVDSWVPEALAPFLCKDKREFNGVSGARLRTVKLRGQISQGLLLPVPEGAAEGDDLSEMLGIQKYEPPIPADLQGIVKGPFPSFVRKTNQERIQNLVAELEEWVEAGLEWEVTEKLDGSSLTAYLFQGEFGVCSRNLDLLETENNSYWKLARENKLEELLRASGRNLAVQGELIGPNVQGNPYGVGAPQLHVFDVYDIDRGGYLTSAERMALLDGAGILHCPVLGTQHLAGASVASLLASAEGKSALKAGTEREGFVFKCLSADVSFKAISNKFLLGEK

SEQ ID NO: 50 - protein, 336 aa, Ignavibacteriaceae bacterium
MRKLATIQIVSDVQPIEGADKIELASILGWKVVIKKGEFEPGDPAIYCEVDSLLPVKPEFEFLRKSSFKRMSDGKEGFRLKTIKLRGQISQGLLLPITALGAHVIDLVPGTDVTNLLEIVKYETPIPAKLAGEVKGPFPGFLSKTDEERVQNLLDELPLYKNSLFYVTEKVDGTSITIYLKDGQFGICSRNLELVENPENTYWKVVRELDIENKLRNLGRNIALQGELLGEGIQKNIYKFKGQTIKFFDAFDIDLYRYFDRKSFFEIMNNFGLETVPVVFDDFTLPESIDEILQMANGKSQLNPDANREGLVFRTTDDKRFSFKAISNNFLLLDEE

SEQ ID NO: 51 - protein, 482 aa, Thermoprotei archaeon
MVPPLKRISEFVWEIPQKYKREMRVPARIFSDEVLLEKMKSDLTLEQAANVACLPGIYKYSIVLPDGHQGYGFPIGGVAAIDYEEGVVSPGGVGYDINCGVRLLRTDLSYEDVKPKIKELINTLFRMVPSGLGSRSHLRLSYGELDEVLASGVEWAVAHGYGWEEDLDRIEERGSMKLADPDKVSDTAKRRGSAQLGTLGSGNHFLEVQVVDKIYNPEVAKVFGITHEGQITVMIHTGSRGLGHQVCSDYLRIMERAVRKYGIRLPDRELAAVPVKSKEGEDYLAAMAAAANFAWTNRQMIMHWVREAFRKVFGQSPEDLGMHLVYDVAHNIAKIEEHTIDGGTRKVVVHRKGATRAFPRGHPAIPAIYRSVGQPVLIPGSMGTASWVLVGTEAAMKITFGSTAHGAGRYLSRAAAVRTWRPRDVAAELERKGVVLRAANARVIAEEAPGAYKDVDRVVEVSHRVGIATKVARLVPIGVTKG

SEQ ID NO: 52 - protein, 383 aa, Klebsiella pneumoniae
MLELYKNLMNLCESSEVAKFFYKDFTGPMDGKFRVFSYHYASYSEWLKPDALECRGIMFEMDGDTPIRVASRPMEKFFNLNENPLTMGIDISDVEYIMDKADGSLVSSYVDDGYLYLKSKTSLYSDQARQASALLNSEEYSSLHQVILELALDGYTVNMEFVSPNNRVVLAYQEPQLFVLNVRNNATGEYIKYDDLYANAKIRPYLINAYGISDPTTWVEGVRELEGVEGYIAVLNTGQRFKVKTEWYSALHHTKDSITSNERLFASVVSANSDDLRSLFAGDEYAIKKISAFEQAYLDYLGKSLELCQSFYDEYRGRARKDYAIAAQKATVNQRHLFGVIMNMYEGTVDVDKLLKDLERVFLKYWAGYVPKEYEKEIELSEE

SEQ ID NO: 53 - protein, 382 aa, Acidobacteria bacterium
MKQMYDNLKALTQKNDMFFSSIQTTPSNKPVEIFSYHIASYSDWLEPDAIECRGIMFDITDKENPVILSRPMEKFFNLGENPLALPEDVLPLVKTIEEKRDGSLISTYLDDGKLYTKSKGSLYSDQANDSNRFLMRSENKDFKQALKTLAELGYTANMEYTSPKNQIVLKYEKQELIVLNIRNTETGDYLTLDDLAELDAENPEHTIYTHIAERFVDYEEVDGMSDEDVERIRDMKGIEGYVLVGQNQRVKLKTDWYVNLHRLKDNINNNRRLVESVVESRTDDLRQLFEHDQGSIDKIKEFEQYVLSKIKSCLAEVRTVYERVKHLDRKHYAINAQRYVDYTPLFSVIMRQFDDYNEENVVENIKQIALKNVDDFIPMHYK

SEQ ID NO: 54 - protein, 334 aa, Salmonella enterica
MFKKYSSLENHYNSKFIEKLYSLGLTGGEWVAREKIHGTNFSLIIERDKVTCAKRTGPILPAEDFFGYEIILKNYADSIKAVQDIMETSAVVTYQVFGEFAGPGIQKNVDYGDKDFYVFDIIVTTESGDVTYVDDYMMESFCNTFKFKMAPLLGRGKFEELIKLPNDLDSVVQDYNFTVDHAGLVDANKCVWNAEAKGEVFTAEGYVLKPCYPSWLPNRNRVAIKCKNSKFSEKKKSDKPIKTKVELSEADNKLMGILACYVTLNRVNNVISKIGEIGPKDFGKVMGLTVQDILEETSREGITLTQADNPSLIKKELVKMVQDVLRPAWIELVS

SEQ ID NO: 55 - protein, 334 aa, Yersinia phage vB_YepM_ZN18
MFKKYSSLENHYNSKFIEKLYSLGLTGGEWVAREKIHGTNFSLIIERDKVTCAKRTGPILPAEDFFGYEIILKNYEDSIKAVQDIMETSAVVSYQVFGEFAGPGIQKNVDYGDKDFYVFDIIVTTESGDVTYVDDYMMESFCNTFKFKMAPLLGRGKFEELIKLPNDLDSVVQDYNFTVDHAGLVDANKCVWKAEAKGEVFTAEGYVLKPCYPSWLHNGNRVAIKCKNSKFSEKKKSDKPIKAKVELSEADNKLVGILACYVTLNRVNNVISKIGEIGPKDFGKVMGLTVQDILEETSREGITLTQADNPSLVKKELVKMVQDVLRPAWIELVS

SEQ ID NO: 56 - RNA, 15 nt, synthetic construct
  source 1..15: mol_type = other RNA; note = Modified with 2'-OCH3 at positions 1, 3, 5, 7, 9, 11, 13, and 15; modified with 2'-F at positions 2, 4, 6, 8, 10, 12, and 14; note = P13
acggggtcactgagt

SEQ ID NO: 57 - RNA, 15 nt, synthetic construct
  source 1..15: mol_type = other RNA; note = Modified with 2'-OCH3 at positions 1, 3, 4, 5, 8, 9, 12, 14, and 15; modified with 2'-F at positions 2, 6, 7, 10, 11, and 13; note = P14
actcagtgaccccgt

SEQ ID NO: 58 - RNA, 11 nt, synthetic construct
  source 1..11: mol_type = other RNA; note = P12; note = Modified with 2'-OCH3 at positions 1, 3, 5, 7, 9, and 11; modified with 2'-F at positions 2, 4, 6, 8, and 10
ggtcactgagt

SEQ ID NO: 59 - DNA, 17 bp, synthetic construct
  source 1..17: mol_type = other DNA; note = P16
aactcagtgaccccgta

SEQ ID NO: 60 - RNA, 38 nt, synthetic construct
  source 1..38: mol_type = other RNA; note = H1; note = All positions from 1 to 38 are modified with 2'-OCH3
agcaagttaagctagaaattaaggctatgttaattaga